European Patent Specification EP 3 260 544 B1, published December 25, 2024. Title: Enzymes and methods for producing omega-3 fatty acids. Applicant: Commonwealth Scientific and Industrial Research Organisation Grains Research and Development Corporation. The sequence listing filed with the application follows.

SEQUENCE LISTING (129 sequences)

SEQ ID NO: 1 - DNA, 825 bp, Micromonas CS-0170
atggctttccccgccgtcgcgaccgctgtcttcggtatctatgcgtacgtgatgtactggtactccgtccccggcgcgggcttcctcgccgagggcaagcaggacgtcgtggcgtggatcggcgatctgtccgtggcgctccccgccaccgccaccgtcctgtacctctccatgtgctacttcggcccgaagatcatggccaagagggaggcgttcgagccgaaggggttcatgctggtgtacaacgcgtaccagaccgtgttcaacatcatcaccgtcgccatcttcatcgctgagctcaaccggctgggcgtgaaggcgtggggcggccgcctgtcgtggtccgatcccaacagcttctacatctgcctcgccatctggctccactacaacaacaagtacctggagctcctcgacaccgtcttcatggtgctgcgcaagaagaacaaccagctcagcttcctccacatctaccaccactgcctcctcatctgggcgtggtggatggtgtgcttcgtcatcaagaacaacgactgcatcgacgcgtactttggcgcctgcatgaacgctggaattcacgtcatcatgtactcctattacctcatggccgcgctgaagatcaagtgcccgtggaagcagtacatcaccatggcgcagatgctccagttcgccatcgtctttgcgcacagctgctacgtcatctacgacgggcactgcccggcgattctgccgtggtcgcagatgttcgtgatgaccaacatgctggtgctgttcgggcagttctacgtgcagacgtacacgaagaagaaggtaaaggccaagtaa

SEQ ID NO: 2 - protein, 274 aa, Micromonas CS-0170
MAFPAVATAVFGIYAYVMYWYSVPGAGFLAEGKQDVVAWIGDLSVALPATATVLYLSMCYFGPKIMAKREAFEPKGFMLVYNAYQTVFNIITVAIFIAELNRLGVKAWGGRLSWSDPNSFYICLAIWLHYNNKYLELLDTVFMVLRKKNNQLSFLHIYHHCLLIWAWWMVCFVIKNNDCIDAYFGACMNAGIHVIMYSYYLMAALKIKCPWKQYITMAQMLQFAIVFAHSCYVIYDGHCPAILPWSQMFVMTNMLVLFGQFYVQTYTKKKVKAK

SEQ ID NO: 3 - DNA, 894 bp, Pyramimonas CS-0140
atggagttcgctcagcctcttgtggctatggcacaggagcagtatgccgcaattgacgcggtggtagcccctgcaattttctcagctaccgacagcatcggttggggtcttaagcccattagcagcgcgacaaaggatcttcctctcgttgagagtccgacgccgctcatactgagcctgttggcctattttgcgatcgtcggctctgggctggtgtaccgcaaagtattccctcgcacagtaaaggggcaagaccccttcctgctgaaggcgctcatgcttgcgcacaacgtgttcctcattggcctcagtctatacatgtgcttgaagcttgtctacgaggcttacgtcaacaagtactccttctggggaaacgcctacaaccccgcacagaccgagatggcgaaggtcatctggattttctacgtctccaagatctatgagttcatggacacgttcatcatgctcttgaagggcaacgtcaaccaggtctctttcctgcatgtgtaccatcatggctccatctctggtatctggtggatgatcacctacgctgcccctggcggtgacgcgtacttctcggcggcgctcaactcgtgggtgcacgtgtgcatgtacacgtactacttcatggcggcggtgctgcccaaggacgagaagaccaagcgcaagtacctctggtggggccgctacctgacccagatgcagatgttccagttcttcatgaacctgctccaggcggtctacctcctctactcctctagcccctaccccaagttcatcgcccagctgctggtggtgtacatggtcacgctgctgatgctcttcggcaacttctactacatgaagcaccacgcgagcaagaagcagaagctggccagcaagaagcagtag

SEQ ID NO: 4 - protein, 297 aa, Pyramimonas CS-0140
MEFAQPLVAMAQEQYAAIDAVVAPAIFSATDSIGWGLKPISSATKDLPLVESPTPLILSLLAYFAIVGSGLVYRKVFPRTVKGQDPFLLKALMLAHNVFLIGLSLYMCLKLVYEAYVNKYSFWGNAYNPAQTEMAKVIWIFYVSKIYEFMDTFIMLLKGNVNQVSFLHVYHHGSISGIWWMITYAAPGGDAYFSAALNSWVHVCMYTYYFMAAVLPKDEKTKRKYLWWGRYLTQMQMFQFFMNLLQAVYLLYSSSPYPKFIAQLLVVYMVTLLMLFGNFYYMKHHASKKQKLASKKQ

SEQ ID NO: 5 - DNA, 804 bp, Pyramimonas CS-0140
atggcgtctattgcgattccggctgcgctggcagggactcttggttatgtgacgtacaatgtcgcaaacccagatattcctgcatccgagaaggtgcctgcttactttatgcaggtcgagtattgggggccaacgattgggaccatcggttatcttctgttcatctactttggtaaacggattatgcaaaacaggagccagccgtttggcctgaagaacgctatgctggtgtacaacttctatcagactttcttcaactcgtactgcatatacctttttgtcacgtcgcaccgcgctcaggggctgaaagtttggggaaacatccccgatatgactgccaacagctgggggatctcacaggtgatctggctgcactacaacaacaagtacgttgagctgctggacacgttcttcatggtcatgcgcaagaagtttgaccagctttcgttcctgcacatttaccatcataccctgttgatctggtcttggttcgtggtgatgaaattggagcccgttggggactgctactttggctctagcgtcaacacgtttgtgcacgtcattatgtactcgtactatggccttgccgcgctcggggtgaattgcttctggaagaagtacattacgcagattcagatgctgcagttctgtatctgcgcttcgcactcgatttataccgcctatgtgcagaacaccgcgttctggttgccttacttgcagctgtgggtgatggtgaacatgttcgtgttgttcgccaacttctatcgcaagcgctacaagagcaagggtgccaagaagcagtaa

SEQ ID NO: 6 - protein, 267 aa, Pyramimonas CS-0140
MASIAIPAALAGTLGYVTYNVANPDIPASEKVPAYFMQVEYWGPTIGTIGYLLFIYFGKRIMQNRSQPFGLKNAMLVYNFYQTFFNSYCIYLFVTSHRAQGLKVWGNIPDMTANSWGISQVIWLHYNNKYVELLDTFFMVMRKKFDQLSFLHIYHHTLLIWSWFVVMKLEPVGDCYFGSSVNTFVHVIMYSYYGLAALGVNCFWKKYITQIQMLQFCICASHSIYTAYVQNTAFWLPYLQLWVMVNMFVLFANFYRKRYKSKGAKKQ

SEQ ID NO: 7 - DNA, 1392 bp, Micromonas CCMP1545
atgtgtcctcctaagaccgatggaagatcttctcctagatctcctctcaccaggtctaagtcatctgctgaggctcttgatgctaaggatgcttctaccgctcctgttgatcttaagacccttgagcctcatgaacttgctgctaccttcgagactagatgggttagggttgaggatgttgagtacgacgtgaccaacttcaaacatcctggtggaagcgtgatcttctacatgcttgctaacactggtgctgatgctactgaggctttcaaagaatttcacatgcgtagcctcaaggcttggaagatgcttagagctttgccttctagacctgctgagatcaagagatctgagtctgaggatgctcctatgcttgaggatttcgctaggtggagagctgaacttgagagggacggattcttcaagccttctatcacccatgttgcttaccgtcttttggagcttcttgctactttcgctcttggaaccgctcttatgtacgctggataccctatcattgctagcgttgtgtacggtgctttcttcggagctagatgtggatgggttcaacatgagggtggacacaactctcttaccggatctgtgtacgtggataagagacttcaggctatgacttgcggattcggactttctaccagcggagagatgtggaaccagatgcataacaagcaccatgctacccctcagaaagttagacacgacatggatcttgataccactcctgctgtggctttcttcaacaccgctgtggaggataatagacctaggggattctctagagcttgggctagacttcaagcttggaccttcgttcctgttacttctggacttctcgttcaggctttctggatctacgttctccatcctagacaggtgctcaggaagaagaactacgaggaagcttcttggatgctcgtttctcacgttgttagaaccgctgttatcaagcttgctaccggatactcttggcctgttgcttactggtggttcactttcggaaactggatcgcttacatgtacctcttcgctcacttctctacttctcacactcacctccctgttgttccatctgacaagcaccttagctgggttaactacgctgttgatcacaccgttgacatcgatccttctcgtggatacgttaactggcttatgggataccttaactgccaggttatccaccatctcttccctgatatgcctcaattcagacagcctgaggtgtcaagaagattcgtccctttcgctaagaagtggggactcaactacaaggtgctctcttactacggtgcttggaaggctactttcagcaacctcgacaaagttggacagcactactacgttaacggaaaggctgagaaggctcactga

SEQ ID NO: 8 - protein, 463 aa, Micromonas CCMP1545
MCPPKTDGRSSPRSPLTRSKSSAEALDAKDASTAPVDLKTLEPHELAATFETRWVRVEDVEYDVTNFKHPGGSVIFYMLANTGADATEAFKEFHMRSLKAWKMLRALPSRPAEIKRSESEDAPMLEDFARWRAELERDGFFKPSITHVAYRLLELLATFALGTALMYAGYPIIASVVYGAFFGARCGWVQHEGGHNSLTGSVYVDKRLQAMTCGFGLSTSGEMWNQMHNKHHATPQKVRHDMDLDTTPAVAFFNTAVEDNRPRGFSRAWARLQAWTFVPVTSGLLVQAFWIYVLHPRQVLRKKNYEEASWMLVSHVVRTAVIKLATGYSWPVAYWWFTFGNWIAYMYLFAHFSTSHTHLPVVPSDKHLSWVNYAVDHTVDIDPSRGYVNWLMGYLNCQVIHHLFPDMPQFRQPEVSRRFVPFAKKWGLNYKVLSYYGAWKATFSNLDKVGQHYYVNGKAEKAH

SEQ ID NO: 9 - DNA, 1449 bp, Ostreococcus lucimarinus
atgtgcgtcgaaacgaccgaaggcacatcgcgaacgatggcgaacgaacgcacgagctcgtcgtcgtcgctgagcgaaggcggaacgccgacggtgacggtcgggatgggaagcgaagacgcggggaagaagactcgaaacgcgagcgtcacggcgtggacgaaagagttggagccgcacgcgatcgcgaagacgttcgaacggcggtacgtgacgatcgaaggcgtggaatacgatgtgacggattttaagcatcccggaggatcggttatttattacatgctgtcgaacacgggagcggacgcgacggaggcttttaaagagtttcattatcggtcgaaaaaggcgcgcaaggcgttggcggcgttgccgcataagccagtggacgcggcgacgcgggaaccgatcgaagatgaggcgatgctgaaggatttcgcgcagtggcgcaaggaattggagcgtgagggattttttaagccctcgccggcgcacgtggcgtatcgattcgccgagctcgcggcgatgttcgcgctcggcacggcgttgatgcacgcgcgttggcacgtcgcttccgtgatcgtgtactcgtgtttcttcggcgcgcgatgcggttgggtgcagcacgagggtgggcacaattcgttgactggaaacatttggtgggacaagcgaatccaagccttcgccgcggggttcggcttggcgtcgagtggcgacatgtggaacaacatgcacaacaagcatcacgcgacgccccaaaaggtgcgacacgatatggatctcgacaccactcccacggtggcgttcttcaactccgcggttgaagaaaatcgcccgcggggattcagtaagttgtggttgcgccttcaagcgtggaccttcgtgcccgtgacgtccggtatggttttgttcttctggatgttcgtcttgcacccgcgtaacgcgctgcgacgcaaaagcttcgaagaagcggcttggatgttttccgcgcacgtcattcgcacggcggttatcaaagccgtcaccggctactcctggatcgcctcgtacggcttgttcgcggcgacgatgtgggcgagcggatgttacttgttcgcgcacttttccacgtctcacacgcacttggatgtcgtgccgagcgataaacacctctcgtgggtgcgatacgccgtcgatcacacgatcgacatcaatccgaacaacagcgtcgtcaactggttgatgggctacttgaactgccaagtcatccatcacctgttcccggatatgcctcagttccgccaacccgaagtctcccgccgattcgtcccgtttgcgaagaagtggaacttaaactacaaggtcttgacgtattatggggcctggaaggcgacgttcggcaacttgaacgacgtcgggaagcactattacgtgcacggatctcagcgcgtcaaatcaaagtcggcgtga

SEQ ID NO: 10 - protein, 482 aa, Ostreococcus lucimarinus
MCVETTEGTSRTMANERTSSSSSLSEGGTPTVTVGMGSEDAGKKTRNASVTAWTKELEPHAIAKTFERRYVTIEGVEYDVTDFKHPGGSVIYYMLSNTGADATEAFKEFHYRSKKARKALAALPHKPVDAATREPIEDEAMLKDFAQWRKELEREGFFKPSPAHVAYRFAELAAMFALGTALMHARWHVASVIVYSCFFGARCGWVQHEGGHNSLTGNIWWDKRIQAFAAGFGLASSGDMWNNMHNKHHATPQKVRHDMDLDTTPTVAFFNSAVEENRPRGFSKLWLRLQAWTFVPVTSGMVLFFWMFVLHPRNALRRKSFEEAAWMFSAHVIRTAVIKAVTGYSWIASYGLFAATMWASGCYLFAHFSTSHTHLDVVPSDKHLSWVRYAVDHTIDINPNNSVVNWLMGYLNCQVIHHLFPDMPQFRQPEVSRRFVPFAKKWNLNYKVLTYYGAWKATFGNLNDVGKHYYVHGSQRVKSKSA

SEQ ID NO: 11 - DNA, 1449 bp, Artificial Sequence
  Codon-optimized nucleotide sequence for production in plants of SEQ ID NO:10
atgtgtgttgagactactgagggaacctctagaactatggctaacgagaggacctcttcttcttcttcactctctgagggtggaactcctactgttactgtgggaatgggatctgaggatgctggaaagaaaaccagaaacgcttctgttactgcttggaccaaagagcttgagcctcacgctatcgctaagaccttcgagagaagatacgttaccatcgagggtgttgagtacgatgtgaccgatttcaaacaccctggtggatctgtgatctactacatgctctctaacactggtgctgatgctactgaggctttcaaagagttccactaccgttctaagaaggctagaaaggctcttgctgctcttcctcacaagcctgttgatgctgctactagagagcctattgaggacgaggctatgcttaaggatttcgctcagtggagaaaagagttggagagagagggattcttcaagccttctcctgctcatgttgcttaccgtttcgctgaactcgctgctatgttcgctcttggaaccgctcttatgcatgctagatggcacgttgctagcgttatcgtgtactcctgtttcttcggagctagatgtggatgggttcaacatgagggtggacacaactctcttaccggaaacatctggtgggataagagaatccaagctttcgctgctggattcggacttgcttcttctggtgacatgtggaacaacatgcacaacaagcaccatgctactcctcagaaagtgagacacgatatggatcttgataccacccctaccgttgctttcttcaactctgctgtggaggaaaacagacctaggggattctctaagctttggctcagacttcaagcttggaccttcgttcctgttacctctggaatggtgctcttcttctggatgttcgttctccatcctagaaacgctctccgtcgtaagtctttcgaagaggctgcttggatgttctctgctcacgttatcagaaccgctgttatcaaggctgttaccggatactcttggatcgctagctacggacttttcgctgctactatgtgggcttctggatgctaccttttcgctcacttctctacttctcacacccacctcgatgttgttccatctgataagcaccttagctgggttaggtacgctgttgatcacaccatcgacatcaaccctaacaactctgttgtgaactggcttatgggataccttaactgccaggttatccaccatctcttccctgatatgcctcaattcagacagcctgaggtgtcaagaagattcgtccctttcgctaagaagtggaacctcaactacaaggtgctcacttactacggtgcttggaaggctactttcggaaacctcaacgatgttggaaagcactactacgttcacggatctcagagagtgaagagcaagagcgcttga

SEQ ID NO: 12 - DNA, 1329 bp, Pyramimonas CS-0140
atgggaaagggaggcaatgctagcgctcctactgcgaagaaggaggtgttgatcgaggggaagttttacgatgtcaccgacttcaggcaccccggtggttcgatcatcaagtttctctcgggttctggtgctgacgccaccgcttcctaccgcgagttccacgttaggtcagcgaaggcagacaagttcttgaagacgctgccctcccgcgaagccactccccaggagctgaagcaggcggttgagttctccaagctcaacccgccctccgcggagagtgcctctgctcccctgaccgaccttgccaaggtggaagcgctgaacaaggacttcgaggctttccgtgagcagctcattcaggagggcttctttaagcccaatatcccgcatgtggtcaagcgcatcacggaagtcgtggcgatgatggccgtagcctcctggatgatggtgcagaccaacgctcttgttgtgaccctcggagttctgatccgcggcattgcacagggccggtgcggttggcttatgcacgagggcggccactatagtcttactgggaagatctccattgataggcgtctgcaggagtcaatttacggattcggctgtggaatgtccggcgcctggtggcgcaaccagcacaacaagcaccacgcaaccccacagaagctgcagcatgacgtcgacctggagacccttcctctgatggctttcaacaacgctgttaccgatagacgcaaggtgaagcctggtagtctccaggctctgtggctcaagtaccaggccttcctcttcttccccgtgacctcccttctggtcggcctcggttggaccaccgtcctccaccccaggcacagcttgcgcaccaagcactatttcgagctgctctgcatggctgctcgttacgcgagtttcgctgctcttttcgctcccaagtacggacttgcaggagctgccgggctctacctcgccaccttcgctgtcgggtgcaactatattttcatcaacttctcggtctctcacactcacctgcccgtgagcggtgcgagcgagtacctgcattgggtcgtgtattcggccatccacaccactaacatcaaatccagcatgctgtgcgattggtggatgtcattcctcaacttccagatcgagcatcacctgttcccttcaatgccccagttccgccacaagattatctccccgcgtgtaaaggccttgtttgagaagcacggtcttgtgtatgatgtgcgcccctattggggggccatggctgacaccttcaagaacttgaatgacgttggcactcacgcatctcactccaaggcgcactag

SEQ ID NO: 13 - protein, 442 aa, Pyramimonas CS-0140
MGKGGNASAPTAKKEVLIEGKFYDVTDFRHPGGSIIKFLSGSGADATASYREFHVRSAKADKFLKTLPSREATPQELKQAVEFSKLNPPSAESASAPLTDLAKVEALNKDFEAFREQLIQEGFFKPNIPHVVKRITEVVAMMAVASWMMVQTNALVVTLGVLIRGIAQGRCGWLMHEGGHYSLTGKISIDRRLQESIYGFGCGMSGAWWRNQHNKHHATPQKLQHDVDLETLPLMAFNNAVTDRRKVKPGSLQALWLKYQAFLFFPVTSLLVGLGWTTVLHPRHSLRTKHYFELLCMAARYASFAALFAPKYGLAGAAGLYLATFAVGCNYIFINFSVSHTHLPVSGASEYLHWVVYSAIHTTNIKSSMLCDWWMSFLNFQIEHHLFPSMPQFRHKIISPRVKALFEKHGLVYDVRPYWGAMADTFKNLNDVGTHASHSKAH

SEQ ID NO: 14 - DNA, 528 bp, Micromonas CS-0170
tgtggtgcatcggccatgattgggggcacggatccttctccaaaaacgccctcgtcaacggcgtcgtcggacacctcacgcactcgccgctgctcgtgcccttttacccgtgggcgtactcgcacaagcagcaccacaggtttcacaaccacgaggtacgggacatgtcgcacccgtggatgtccaaggaggagtacgcggacgtgaaccccgtcgtgagggcgctggcgctggacggttggtggggaaccttcctcggctttcccgggtacctcctcctggaaccgcagtgggccgggacggacgggtgccacttcaacccgaactccaggctcttcgacagggcgcccaaggatgagcgggtgaagtgcgcggtttccaccgtggcgtgcgcggcgtttctcggcgcgtccttcgtcgcgtgcgactcgaaccccgttcactggttcgctcagtacttggcgccgtacttgtgcttctcgtggtggctcttcaccgtgacatacttacagcacaacgacgaggaca

SEQ ID NO: 15 - protein, 175 aa, Micromonas CS-0170
WCIGHDWGHGSFSKNALVNGVVGHLTHSPLLVPFYPWAYSHKQHHRFHNHEVRDMSHPWMSKEEYADVNPVVRALALDGWWGTFLGFPGYLLLEPQWAGTDGCHFNPNSRLFDRAPKDERVKCAVSTVACAAFLGASFVACDSNPVHWFAQYLAPYLCFSWWLFTVTYLQHNDED

SEQ ID NO: 16 - DNA, 1461 bp, Micromonas RCC299
atgaccgccgtcggcggcgggcgtcgacactcccgcgccgcgcgtcccgagcggactcgagaccgtcggaagcgctcgtcggattccacagagtcggattccgtcgtctcccggacacccggcgacgtacctcccgccgcgctcgttcacgcgatgcccgcgatgatgacctcatccacctgtctgcgggccacgtcgccccggatggaatcgacacgccgcggctccctccgcgtcgtcgacgccgcggcgcccgcacgcaccggcgcatccaagacgggtcggtccgtcccgcgtcaactcccccgcgccatttccgcgccgacgacgaacctcggaaccgcggacgcgccaactcccgccgccggtcccgtgccgtccctccgagagctgcgcgcatccatcccgaaggagtgcttcgagcccgacctgggggagtcgctcaagtacgccgcgtacgatctcgccgcgctcgccgcgtgcttcggcgtcatctccccgcacgtggtggaccacccgtggctgttaccgctgtacgcgcccctcacgggcaccgtcatgtggatgaacttcgtcgtcggccacgactgcgggcacggctccttctccaaatcctccgtcgtcaacggcgtcgtcggccacctcacgcactcgccgctgctcgtgcccttctacccgtgggcgtactcgcacaagcagcaccacaggtttcacaaccaccaggtaaaggacatgtcgcacccgtggatgactgcagaggagtacgccgaggtgaaccccatcgtccgggctctggcgcttgacgggtggtggggaaccttcctcggctttcccgggtacctcctcctggaaccgcggtgggccgggacggacgggtgccacttcaacccacaatccaggctcttcgacagggcgcccaaggacgagcgggtgaagtgcgcggtttccaccgtggcgtgcgcggcgtttctcggcgcgtccttcgtcgcgtgcgactcgaacccggcgcactggttcgctcagtacttggcgccgtacttgtgcttctcgtggtggctcttcaccgtgacctacctccagcaccacgactacgacacaacgacgtacgaagagggccagtgggagtacgtgctggggggtttggagacgatcgaccgcgagtttgggcacggcgtggacgagctgacgcatcacatcaccgactgccacgtcgcgcaccacatgttctcggacatgccccactaccgcctgcccgcggcgaccgccggggtgcgatcggtgctggagccccgtgggttgtacaagcgacgggacacgcgggatttcgtgacgaaggtgttcgagttgcacggggacgtcgggcactgcgtggagagcgaggcgggggtgaggccgagggcgacgcgcgacgagtgcgcggcggcgttcaacggcgaggagtggcgcgaggttcgcaagtag

SEQ ID NO: 17 - protein, 486 aa, Micromonas RCC299
MTAVGGGRRHSRAARPERTRDRRKRSSDSTESDSVVSRTPGDVPPAALVHAMPAMMTSSTCLRATSPRMESTRRGSLRVVDAAAPARTGASKTGRSVPRQLPRAISAPTTNLGTADAPTPAAGPVPSLRELRASIPKECFEPDLGESLKYAAYDLAALAACFGVISPHVVDHPWLLPLYAPLTGTVMWMNFVVGHDCGHGSFSKSSVVNGVVGHLTHSPLLVPFYPWAYSHKQHHRFHNHQVKDMSHPWMTAEEYAEVNPIVRALALDGWWGTFLGFPGYLLLEPRWAGTDGCHFNPQSRLFDRAPKDERVKCAVSTVACAAFLGASFVACDSNPAHWFAQYLAPYLCFSWWLFTVTYLQHHDYDTTTYEEGQWEYVLGGLETIDREFGHGVDELTHHITDCHVAHHMFSDMPHYRLPAATAGVRSVLEPRGLYKRRDTRDFVTKVFELHGDVGHCVESEAGVRPRATRDECAAAFNGEEWREVRK

SEQ ID NO: 18 - DNA, 1461 bp, Artificial Sequence
  Codon-optimized nucleotide sequence for production in plants of SEQ ID NO:17
atgactgctgttggaggtggaagaaggcattctagagctgctagacctgagagaaccagggatcgtagaaagagatcttctgactctaccgagtctgattctgtggtttctaggacccctggtgatgttcctcctgctgctcttgttcatgctatgcctgctatgatgacctcttctacctgccttagagctacttctcctaggatggaatctaccagaaggggatctctcagagttgttgacgctgctgctccagctagaactggtgcttctaagaccggaagatctgttcctagacagctccctagagctatctctgctcctactactaaccttggaaccgctgatgctcctactcctgctgctggacctgttccttctcttagagagcttagggctagcatccctaaagagtgcttcgagcctgatcttggagagtctctcaagtacgctgcttacgatcttgctgctctcgctgcttgtttcggagttatctctcctcacgttgttgatcatccttggcttctcccactttacgctcctcttaccggaactgtgatgtggatgaacttcgttgttggacatgattgcggacacggatctttctctaagtctagcgtggttaacggtgttgttggacaccttacccactctcctcttctcgttcctttctacccttgggcttactctcataagcagcaccacagattccataaccaccaggtgaaggatatgtctcacccttggatgactgctgaggaatacgctgaggttaaccctattgtgagggctcttgctcttgatggatggtggggaactttccttggattccctggataccttcttcttgagcctagatgggctggaactgatggatgtcacttcaaccctcagtctagacttttcgacagggctcctaaggatgaacgtgttaagtgcgctgtttctactgttgcttgcgctgctttccttggagcttctttcgtggcttgcgattctaaccctgctcattggttcgctcagtaccttgctccttacctttgcttctcttggtggctcttcactgttacttacctccagcaccacgattacgataccactacctacgaggaaggacagtgggaatacgttcttggaggactcgagactatcgatagagaatttggacacggtgttgatgagcttactcaccacatcactgattgtcacgtggctcaccacatgttctctgacatgcctcattacagacttccagctgctactgctggtgttagatctgttctcgagcctagaggactctacaagagaagagacaccagggatttcgttaccaaggtgttcgagcttcatggtgatgttggacactgcgttgagtctgaagctggtgttaggcctagagctactagagatgagtgcgctgctgcttttaatggtgaagagtggagggaagttaggaagtga

SEQ ID NO: 19 - DNA, 1389 bp, Micromonas CCMP1545
atgacggcggcgacgacgctctcgcgcgcgtcctccgtcgtcggcgtcggcgcaggcgccacgtcgaggcgtccggtcgatcgcgccgtctccgccgtcgcgacgtcctcctcgtattcgcgccgcgcgcgccgcgtcgcgaccgtccgcgcggcgtccagccgcacgtcgtcctccgcgacgacgacgacgacgacgacgacgcgctccgctctggccatggagaccccgtccacgacgacgacggacgcggacgacgacgacgacaagaccggcgtcgtcccgtcgctccgagagctccgagccgcgatccccgcggagtgcttcgtcccgtgcctgagggagtcgatgaagtacgccgcgatcgacctcggtctcctcgccgcctgcttcggtctgtggtctccgctcgtggtggataacccgtggatgctcccgctgtacgcccccgtcaccgggacgatcatgtggatgtgcttcgtcgtcgggcacgactgcgggcacggcagtttcaggtgcgtcagttctacaaacgtcgagaacaagtggatcaacggcgtcgtcggtcacgcgacgcactcgccgctgctcgtgccgttctacccgtgggcgtactcgcacaagcagcaccaccggtttcataaccacgaggagaaggacatgtcgcacccgtggatgagcgcggagcggtacaaggacacgaacgcgatcgttcggtgcgcggcgggcggctcggtttctggtttttggttcctcgcgctcgatcacccatggggcgcgtttctcggcttccccgggtatctcctcctcgagccaaagtggagcagcacggacggctcgcacttcaacccggccggtcgtctgttcgaccgcgcccccaaggacgaacgtctcaagtgcgcggtctcgacggtcgcgtgcgcggcgttcctcctcgcgacgttcgccgcgtgcgacggccccgcgcagtgggcgacgcagtacctcgcgccgtatctgtgcttctcgtggtggctcttcacggtgacctacctccagcaccacgaccacgacacgaagacgtacaaggaaggcgagtgggagtacgtcttggggggattagagacgatcgatcgcgagttcgggtacggcgtggacgaggcgacgcatcacatcacggactgccacgtcgcgcaccacatgttttcggacatgccgcactacaacttggagaaggccaccgcgggggtgcggggcgtgctcgagcccaggggactgtataagaagagggacacgagggatttcgcgacgaagatttttgggttgcacaaagacgtcgggcactgcgtcgagccggaccggccgcgggcgacgaaggaggagctcgtgaaggcgttggggcgggagtga

SEQ ID NO: 20 - protein, 462 aa, Micromonas CCMP1545
MTAATTLSRASSVVGVGAGATSRRPVDRAVSAVATSSSYSRRARRVATVRAASSRTSSSATTTTTTTTRSALAMETPSTTTTDADDDDDKTGVVPSLRELRAAIPAECFVPCLRESMKYAAIDLGLLAACFGLWSPLVVDNPWMLPLYAPVTGTIMWMCFVVGHDCGHGSFRCVSSTNVENKWINGVVGHATHSPLLVPFYPWAYSHKQHHRFHNHEEKDMSHPWMSAERYKDTNAIVRCAAGGSVSGFWFLALDHPWGAFLGFPGYLLLEPKWSSTDGSHFNPAGRLFDRAPKDERLKCAVSTVACAAFLLATFAACDGPAQWATQYLAPYLCFSWWLFTVTYLQHHDHDTKTYKEGEWEYVLGGLETIDREFGYGVDEATHHITDCHVAHHMFSDMPHYNLEKATAGVRGVLEPRGLYKKRDTRDFATKIFGLHKDVGHCVEPDRPRATKEELVKALGRE

SEQ ID NO: 21 - DNA, 792 bp, Isochrysis galbana
atggccctcgcaaacgacgcgggagagcgcatctgggcggctgtgaccgacccggaaatcctcattggcaccttctcgtacttgctactcaaaccgctgctccgcaattccgggctggtggatgagaagaagggcgcatacaggacgtccatgatctggtacaacgttctgctggcgctcttctctgcgctgagcttctacgtgacggcgaccgccctcggctgggactatggtacgggcgcgtggctgcgcaggcaaaccggcgacacaccgcagccgctcttccagtgcccgtccccggtttgggactcgaagctcttcacatggaccgccaaggcattctattactccaagtacgtggagtacctcgacacggcctggctggtgctcaagggcaagagggtctcctttctccaggccttccaccactttggcgcgccgtgggatgtgtacctcggcattcggctgcacaacgagggcgtatggatcttcatgtttttcaactcgttcattcacaccatcatgtacacctactacggcctcaccgccgccgggtataagttcaaggccaagccgctcatcaccgcgatgcagatctgccagttcgtgggcggcttcctgttggtctgggactacatcaacgtcccctgcttcaactcggacaaagggaagttgttcagctgggctttcaactatgcatacgtcggctcggtcttcttgctcttctgccactttttctaccaggacaacttggcaacgaagaaatcggccaaggcgggcaagcagctctag

SEQ ID NO: 22 - protein, 263 aa, Isochrysis galbana
MALANDAGERIWAAVTDPEILIGTFSYLLLKPLLRNSGLVDEKKGAYRTSMIWYNVLLALFSALSFYVTATALGWDYGTGAWLRRQTGDTPQPLFQCPSPVWDSKLFTWTAKAFYYSKYVEYLDTAWLVLKGKRVSFLQAFHHFGAPWDVYLGIRLHNEGVWIFMFFNSFIHTIMYTYYGLTAAGYKFKAKPLITAMQICQFVGGFLLVWDYINVPCFNSDKGKLFSWAFNYAYVGSVFLLFCHFFYQDNLATKKSAKAGKQL

SEQ ID NO: 23 - DNA, 1284 bp, Pavlova salina
atgggacgcggcggagacagcagtgggcaggcgcatccggcggcggagctggcggtcccgagcgaccgcgcggaggtgagcaacgctgacagcaaagcgctgcacatcgtgctgtatggcaagcgcgtggatgtgaccaagttccaacgcacgcacccgggtggtagcaaggtcttccggatcttccaggaccgcgatgcgacggagcagttcgagtcctaccactcgaagcgcgcgatcaagatgatggagggcatgctcaagaagtctgaggatgctcccgccgacacgcccttgccctcccagtcaccgatggggaaggacttcaaggcgatgatcgagcggcacgttgcagcgggttactacgatccatgcccgctcgatgagctgttcaagctcagcctcgtgctcctcccgacctttgcgggcatgtacatgctcaaggcgggcgtcggctccccgctctgcggcgccctcatggtgagctttggctggtacctcgatggctggctcgcgcacgactatctgcaccactccgtcttcaaggggtccgtcgcacgcaccgtcgggtggaacaacgcggcgggctacttcctcggcttcgtgcaggggtatgcggtcgagtggtggcgcgcgcggcataacacgcaccacgtgtgcaccaatgaggacggctcggaccccgacatcaaaacggcgccgctgctcatatacgtgcgcaacaagccgagcatcgccaagcgcctgaacgccttccagcgctaccagcagtactactatgtgccggtgatggcaatcctcgacctgtactggcggctcgagtcgatcgcctacgtcgcgatgcgcctgccgaagatgctgccgcaggccctcgcactcgtcgcgcactacgccatcgtcgcgtgggtctttgcgggcaactaccacctgctcccgctcgtgacggttctgcgcgggtttggcactgggatcaccgttttcgcgacgcactacggtgaggacattctcgacgcggaccaggtgcgtcacatgacgctcgtcgagcagacggcactcacctcgcgcaacatctcgggcggctggctcgtgaacgtgctcaccggcttcatctcactgcagacggagcaccacctgttcccgatgatgccaaccggcaacctcatgactatccagcccgaggtgcgcgccttcttcaagaagcacggacttgagtaccgcgagggcaacctcattgagtgcgtgcggcagaacatccgtgcgcttgcattcgagcacctgctttga

SEQ ID NO: 24 - protein, 427 aa, Pavlova salina
MGRGGDSSGQAHPAAELAVPSDRAEVSNADSKALHIVLYGKRVDVTKFQRTHPGGSKVFRIFQDRDATEQFESYHSKRAIKMMEGMLKKSEDAPADTPLPSQSPMGKDFKAMIERHVAAGYYDPCPLDELFKLSLVLLPTFAGMYMLKAGVGSPLCGALMVSFGWYLDGWLAHDYLHHSVFKGSVARTVGWNNAAGYFLGFVQGYAVEWWRARHNTHHVCTNEDGSDPDIKTAPLLIYVRNKPSIAKRLNAFQRYQQYYYVPVMAILDLYWRLESIAYVAMRLPKMLPQALALVAHYAIVAWVFAGNYHLLPLVTVLRGFGTGITVFATHYGEDILDADQVRHMTLVEQTALTSRNISGGWLVNVLTGFISLQTEHHLFPMMPTGNLMTIQPEVRAFFKKHGLEYREGNLIECVRQNIRALAFEHLL

SEQ ID NO: 25 - DNA, 1278 bp, Pavlova salina
atgccgccgcgcgatagctactcgtacgccgccccgccgtcggcccagctgcacgaggtcgataccccgcaggagcatgataagaaggagctcgtcatcggtgaccgcgcgtacgacgtgaccaactttgtgaagcgccacccgggtggcaagatcatcgcataccaggttggcacagatgcgacggacgcgtacaagcagttccatgtgcggtctgccaaggcggacaagatgctcaagtcgctgccttcgcgcccggtgcacaagggctactcgccccgccgcgctgacctcattgccgacttccaggagttcaccaagcagctggaggcggagggcatgtttgagccgtcgctgccgcacgtggcataccgcctggcggaggtgatcgcgatgcacgtggccggcgccgcgctcatctggcacgggtacaccttcgcgggcattgccatgctcggcgttgtgcagggccgctgcggctggctcatgcacgagggcggccactactcgctcacgggcaacattgcttttgaccgtgccatccaagtcgcgtgctacggccttggctgcggcatgtcgggcgcgtggtggcgcaaccagcacaacaagcaccacgcgacgccgcagaagttgcagcacgacgtcgacctcgacaccctcccgctcgtcgccttccacgagcggatagccgccaaggtgaagagccccgcgatgaaggcgtggcttagtatgcaggcgaagctcttcgcgccagtgaccacgctgctggtcgcgctgggctggcagctgtacctgcacccgcgccatatgctgcgcaccaagcactacgacgagctcgcgatgctcggcattcgctacggccttgtcggctacctcgcggcgaactacggcgcggggtacgtgctcgcgtgctacctgctgtacgtgcagctcggcgccatgtacatcttctgcaactttgccgtgtcgcacacacacctgccggttgtcgagcctaacgagcacgcaacgtgggtggagtacgccgcgaaccacacgaccaactgctcgccctcgtggtggtgcgactggtggatgtcgtacctcaactaccagatcgagcaccacctctacccgtccatgccgcagttccgccacccgaagattgcgccgcgggtgaagcagctcttcgagaagcacggcctgcactacgacgtgcgtggctacttcgaggccatggcggacacgtttgccaaccttgacaacgtcgcgcacgcgccggagaagaagatgcagtga

SEQ ID NO: 26 - protein, 425 aa, Pavlova salina
MPPRDSYSYAAPPSAQLHEVDTPQEHDKKELVIGDRAYDVTNFVKRHPGGKIIAYQVGTDATDAYKQFHVRSAKADKMLKSLPSRPVHKGYSPRRADLIADFQEFTKQLEAEGMFEPSLPHVAYRLAEVIAMHVAGAALIWHGYTFAGIAMLGVVQGRCGWLMHEGGHYSLTGNIAFDRAIQVACYGLGCGMSGAWWRNQHNKHHATPQKLQHDVDLDTLPLVAFHERIAAKVKSPAMKAWLSMQAKLFAPVTTLLVALGWQLYLHPRHMLRTKHYDELAMLGIRYGLVGYLAANYGAGYVLACYLLYVQLGAMYIFCNFAVSHTHLPVVEPNEHATWVEYAANHTTNCSPSWWCDWWMSYLNYQIEHHLYPSMPQFRHPKIAPRVKQLFEKHGLHYDVRGYFEAMADTFANLDNVAHAPEKKMQ

SEQ ID NO: 27 - DNA, 801 bp, Emiliania huxleyi CCMP1516
atgctcgatcgcgcctcgtccgacgcggccatctggtctgcggtgtccgatccggaaatcctgatcggcactttctcctacctgctgctcaagccgctgctacgcaactcagggctcgtggacgagcggaaaggcgcctaccggacctcgatgatctggtacaacgtggtgctcgcgctcttctccgcgacgagcttctacgtgactgcgaccgcgctcgggtgggacaagggcaccggcgagtggctccgcagtctcacgggcgacagcccgcagcagctgtggcaatgcccgtcgagggtatgggactccaagctgttcctgtggacggccaaggccttctactactcaaagtacgtggagtacctcgacacggcgtggctcgtcctcaaggggaagaaggtctccttcctgcagggcttccaccactttggcgcgccgtgggacgtgtacctgggcattcggctgaagaacgagggcgtgtggatcttcatgttcttcaactcgttcatccacacggtcatgtacacgtactacggcctcaccgccgcgggctacaagatccgcggcaagccgatcatcaccgcgatgcaaataagccagttcgtcggcggctttgtcctagtgtgggactacatcaacgtgccgtgcttccacgccgacgccgggcaggtcttcagctgggtctttaactatgcttacgtcggctccgtctttctgctgttctgccacttcttctacatggacaacatcgcgaaggccaaggccaagaaggccgtcgctacccgcaaggcgctgtga

SEQ ID NO: 28 - protein, 266 aa, Emiliania huxleyi CCMP1516
MLDRASSDAAIWSAVSDPEILIGTFSYLLLKPLLRNSGLVDERKGAYRTSMIWYNVVLALFSATSFYVTATALGWDKGTGEWLRSLTGDSPQQLWQCPSRVWDSKLFLWTAKAFYYSKYVEYLDTAWLVLKGKKVSFLQGFHHFGAPWDVYLGIRLKNEGVWIFMFFNSFIHTVMYTYYGLTAAGYKIRGKPIITAMQISQFVGGFVLVWDYINVPCFHADAGQVFSWVFNYAYVGSVFLLFCHFFYMDNIAKAKAKKAVATRKAL

SEQ ID NO: 29 - DNA, 801 bp, Artificial Sequence
  Codon-optimized nucleotide sequence for production in plants of SEQ ID NO:28
atgcttgatagagcttcatctgatgctgctatttggagcgctgtttctgatcctgagatccttatcggaaccttctcttaccttttgcttaagcctctcctcagaaactctggacttgtggatgagagaaagggagcttaccgtacttctatgatctggtacaacgttgttcttgctcttttctctgctacctctttctacgttactgctactgctcttggatgggataagggaactggtgagtggcttagatctcttactggtgattctcctcaacaactttggcagtgcccttctagagtttgggacagcaaactcttcttgtggactgctaaagccttctactactccaagtacgttgagtaccttgatactgcttggcttgttctcaagggaaagaaggtttcattcctccagggattccatcatttcggtgctccatgggatgtttaccttggaatcaggcttaagaacgagggagtttggatcttcatgttcttcaacagcttcatccacactgttatgtacacttactacggacttactgctgctggatacaagatcagaggaaagcctatcatcaccgctatgcaaatctctcaattcgttggtggattcgttcttgtgtgggactacatcaacgttccttgtttccatgctgatgctggacaagttttctcttgggtgttcaactacgcttatgtgggatctgttttccttcttttctgccacttcttctacatggacaacattgctaaggctaaggctaaaaaggctgttgctaccagaaaggctctttga

SEQ ID NO: 30 - protein, 456 aa, Ostreococcus tauri
MCVETENNDGIPTVEIAFDGERERAEANVKLSAEKMEPAALAKTFARRYVVIEGVEYDVTDFKHPGGTVIFYALSNTGADATEAFKEFHHRSRKARKALAALPSRPAKTAKVDDAEMLQDFAKWRKELERDGFFKPSPAHVAYRFAELAAMYALGTYLMYARYVVSSVLVYACFFGARCGWVQHEGGHSSLTGNIWWDKRIQAFTAGFGLAGSGDMWNSMHNKHHATPQKVRHDMDLDTTPAVAFFNTAVEDNRPRGFSKYWLRLQAWTFIPVTSGLVLLFWMFFLHPSKALKGGKYEELVWMLAAHVIRTWTIKAVTGFTAMQSYGLFLATSWVSGCYLFAHFSTSHTHLDVVPADEHLSWVRYAVDHTIDIDPSQGWVNWLMGYLNCQVIHHLFPSMPQFRQPEVSRRFVAFAKKWNLNYKVMTYAGAWKATLGNLDNVGKHYYVHGQHSGKTA

SEQ ID NO: 31 - protein, 8 aa, Artificial Sequence
  Elongase consensus domain 1
  MISC_FEATURE (2)..(6): X = Any amino acid
KXXXXXDT

SEQ ID NO: 32 - protein, 5 aa, Artificial Sequence
  Elongase consensus domain 2
  MISC_FEATURE (3)..(3): X = any amino acid
MYXYY

SEQ ID NO: 33 - protein, 8 aa, Artificial Sequence
  Elongase consensus domain 3
KIYEFVDT

SEQ ID NO: 34 - protein, 7 aa, Artificial Sequence
  Elongase consensus domain 4
VHVCMYT

SEQ ID NO: 35 - protein, 7 aa, Artificial Sequence
  Elongase consensus domain 5
YLELLDT

SEQ ID NO: 36 - protein, 5 aa, Artificial Sequence
  Elongase consensus domain 6
MYSYY

SEQ ID NO: 37 - protein, 10 aa, Artificial Sequence
  Desaturase consensus domain 1
WKNMHNKHHA

SEQ ID NO: 38 - protein, 8 aa, Artificial Sequence
  Desaturase consensus domain 2
HHLFPSMP

SEQ ID NO: 39 - protein, 8 aa, Artificial Sequence
  Desaturase consensus domain 3
WCIGHDCG

SEQ ID NO: 40 - protein, 10 aa, Artificial Sequence
  Desaturase consensus domain 4
TFLQHHDEDM

SEQ ID NO: 41 - DNA, 37 bp, Artificial Sequence
  Oligonucleotide primer
atttaggtgacactatagttttttttttttttttttv

SEQ ID NO: 42 - DNA, 23 bp, Artificial Sequence
  Oligonucleotide primer
  misc_feature (7)..(7): n= inosine
  misc_feature (14)..(14): n= inosine
aagwwcnksgarynsytcgacac

SEQ ID NO: 43 - DNA, 20 bp, Artificial Sequence
  Oligonucleotide primer
  misc_feature: n = inosine
  misc_feature (2)..(3): n = inosine
  misc_feature (5)..(5): n = inosine
annmnrtartasgtgtacat

SEQ ID NO: 44 - DNA, 21 bp, Artificial Sequence
  Oligonucleotide primer
gaacaacgactgcatcgacgc

SEQ ID NO: 45 - DNA, 23 bp, Artificial Sequence
  Oligonucleotide primer
cgactggagcacgaggacactga

SEQ ID NO: 46 - DNA, 23 bp, Artificial Sequence
  Oligonucleotide primer
ttgcgcagcaccataaagacggt

SEQ ID NO: 47 - DNA, 26 bp, Artificial Sequence
  Oligonucleotide primer
ggacactgacatggactgaaggagta

SEQ ID NO: 48 - DNA, 22 bp, Artificial Sequence
  Oligonucleotide primer
caggcgacgcgcgccagagtcc

SEQ ID NO: 49 - DNA, 26 bp, Artificial Sequence
  Oligonucleotide primer
ttattagttacttggcctttaccttc

SEQ ID NO: 50 - DNA, 23 bp, Artificial Sequence
  Oligonucleotide primer
  misc_feature (18)..(18): n = inosine
aaratmtaygagttygtngatac

SEQ ID NO: 51 - DNA, 25 bp, Artificial Sequence
  Oligonucleotide primer
  misc_feature (3)..(3): n = inosine
tangtgtacatgcacacrtgwaccc

SEQ ID NO: 52 - DNA, 22 bp, Artificial Sequence
  Oligonucleotide primer
ttcgtggatacgttcatcatgc

SEQ ID NO: 53 - DNA, 23 bp, Artificial Sequence
  Oligonucleotide primer
agttgagcgccgccgagaagtac

SEQ ID NO: 54 - DNA, 22 bp, Artificial Sequence
  Oligonucleotide primer
acctggttgacgttgcccttca

SEQ ID NO: 55 - DNA, 21 bp, Artificial Sequence
  Oligonucleotide primer
gctatggagttcgctcagcct

SEQ ID NO: 56 - DNA, 26 bp, Artificial Sequence
  Oligonucleotide primer
ttactactgcttcttgctggccagct

SEQ ID NO: 57 - DNA, 22 bp, Artificial Sequence
  Oligonucleotide primer
artayytsgarytrytggayac

SEQ ID NO: 58 - DNA, 21 bp, Artificial Sequence
  Oligonucleotide primer
catkarrtartasgagtacat

SEQ ID NO: 59 - DNA, 22 bp, Artificial Sequence
  Oligonucleotide primer
catcatccctgttgatctggtc

SEQ ID NO: 60 - DNA, 23 bp, Artificial Sequence
  Oligonucleotide primer
ccagatcaacagggtatgatggt

SEQ ID NO: 61 - DNA, 27 bp, Artificial Sequence
  Oligonucleotide primer
cgaaagctggtcaaacttcttgcgcat

SEQ ID NO: 62 - DNA, 27 bp, Artificial Sequence
  Oligonucleotide primer
aacatggcgtctattgcgattccggct

SEQ ID NO: 63 - DNA, 27 bp, Artificial Sequence
  Oligonucleotide primer
ttattactgcttcttggcacccttgct

SEQ ID NO: 64 - DNA, 31 bp, Artificial Sequence
  Oligonucleotide primer
  misc_feature (23)..(23): n = inosine
ggtggaagaacaagcacaacrdncaycaygc

SEQ ID NO: 65 - DNA, 24 bp, Artificial Sequence
  Oligonucleotide primer
  misc_feature (16)..(16): n = inosine
gggcatcgtggggwanarrtgrtg

SEQ ID NO: 66 - DNA, 20 bp, Artificial Sequence
  Oligonucleotide primer
agcgagtacctgcattgggt

SEQ ID NO: 67 - DNA, 27 bp, Artificial Sequence
  Oligonucleotide primer
atagtgcttggtgcgcaagctgtgcct

SEQ ID NO: 68 - DNA, 25 bp, Artificial Sequence
  Oligonucleotide primer
caccatgggaaagggaggcaatgct

SEQ ID NO: 69 - DNA, 25 bp, Artificial Sequence
  Oligonucleotide primer
ttactagtgcgccttggagtgagat

SEQ ID NO: 70 - DNA, 25 bp, Artificial Sequence
  Oligonucleotide primer
  misc_feature (20)..(20): n = inosine
  misc_feature (23)..(23): n = inosine
tgtggtgcatcggccayganksngg

SEQ ID NO: 71 - DNA, 28 bp, Artificial Sequence
  Oligonucleotide primer
  misc_feature (20)..(20): n = inosine
  misc_feature (26)..(26): n = inosine
tgtcctcgtcgttgtgctgnarrwangt

SEQ ID NO: 72 - DNA, 1344 bp, Pavlova salina
atgcctccgagcgcggcgaagcagatgggcgcgagcacgggcgtgcatgcgggcgtcacagattcgtcggccttcacgcgcaaggatgtcgccgacaggccggacctcacgatcgtgggtgacagcgtgtacgatgcgaaggcgttccgctccgagcatccgggtggcgcgcactttgtgtcgctgttcggcgggcgcgatgccacggaggcgttcatggagtaccaccggcgcgcctggcccaagtcgcgcatgtcgcgcttccacgtcggctctctggcatcgaccgaggagcccgtcgccgccgatgagggctacctccagctgtgcgctcgcatcgccaagatggtgccgtcggtcagcagcgggttcgcgccggcgtcgtactgggtgaaggccgggctgatcctcggctccgcgatcgcgctcgaggcgtacatgctgtacgcgggcaagcgcctgctcccgtcgatcgtgctcgggtggctgtttgcgctgattggcctgaacatccagcacgatgccaaccacggcgcgctctccaagtcggcctcggtcaacctggcgctcgggttgtgccaggactggatcggcgggagcatgatcctctggctgcaggagcacgttgtcatgcaccacttgcacaccaacgacgttgacaaggacccggaccagaaggcgcacggcgccctgcggctcaagccgaccgacgcgtggagcccgatgcactggctgcagcacctctacctgctgcctggggagacgatgtacgccttcaagctgctgtttctcgacatcagcgagctggtgatgtggcggtgggagggcgagcccatcagcaagctggccgggtacctcttcatgccctcgctgctcctcaagctcaccttctgggcgcgctttgtcgcgctgccgctgtacctcgcgcccagcgtgcacacggcggtgtgcatcgcggcgacggtaatgacggggagcttctacctcgccttcttcttcttcatctcgcacaacttcgagggcgtggcgagcgtcggaccggacggcagcatcaccagcatgacgcgcggcgcatccttcctcaagcggcaggccgagacctcgtccaacgtgggcggcccgctgctcgccacgctcaacggcggcctcaactaccaaatcgagcaccacctcttccccagggtgcaccacggcttctaccctcgcctcgcgccgttggtcaaggcggagctcgaggcgcgcggcattgagtacaagcactaccccaccatatggagcaacctggcatccacgctgaggcacatgtacgcgctcggccgcaggccgcgcagcaaggcggagtga

SEQ ID NO: 73 - protein, 447 aa, Pavlova salina
MPPSAAKQMGASTGVHAGVTDSSAFTRKDVADRPDLTIVGDSVYDAKAFRSEHPGGAHFVSLFGGRDATEAFMEYHRRAWPKSRMSRFHVGSLASTEEPVAADEGYLQLCARIAKMVPSVSSGFAPASYWVKAGLILGSAIALEAYMLYAGKRLLPSIVLGWLFALIGLNIQHDANHGALSKSASVNLALGLCQDWIGGSMILWLQEHVVMHHLHTNDVDKDPDQKAHGALRLKPTDAWSPMHWLQHLYLLPGETMYAFKLLFLDISELVMWRWEGEPISKLAGYLFMPSLLLKLTFWARFVALPLYLAPSVHTAVCIAATVMTGSFYLAFFFFISHNFEGVASVGPDGSITSMTRGASFLKRQAETSSNVGGPLLATLNGGLNYQIEHHLFPRVHHGFYPRLAPLVKAELEARGIEYKHYPTIWSNLASTLRHMYALGRRPRSKAE

SEQ ID NO: 74 - DNA, 1563 bp, Arabidopsis thaliana
atggcgattttggattctgctggcgttactacggtgacggagaacggtggcggagagttcgtcgatcttgataggcttcgtcgacggaaatcgagatcggattcttctaacggacttcttctctctggttccgataataattctccttcggatgatgttggagctcccgccgacgttagggatcggattgattccgttgttaacgatgacgctcagggaacagccaatttggccggagataataacggtggtggcgataataacggtggtggaagaggcggcggagaaggaagaggaaacgccgatgctacgtttacgtatcgaccgtcggttccagctcatcggagggcgagagagagtccacttagctccgacgcaatcttcaaacagagccatgccggattattcaacctctgtgtagtagttcttattgctgtaaacagtagactcatcatcgaaaatcttatgaagtatggttggttgatcagaacggatttctggtttagttcaagatcgctgcgagattggccgcttttcatgtgttgtatatccctttcgatctttcctttggctgcctttacggttgagaaattggtacttcagaaatacatatcagaacctgttgtcatctttcttcatattattatcaccatgacagaggttttgtatccagtttacgtcaccctaaggtgtgattctgcttttttatcaggtgtcactttgatgctcctcacttgcattgtgtggctaaagttggtttcttatgctcatactagctatgacataagatccctagccaatgcagctgataaggccaatcctgaagtctcctactacgttagcttgaagagcttggcatatttcatggtcgctcccacattgtgttatcagccaagttatccacgttctgcatgtatacggaagggttgggtggctcgtcaatttgcaaaactggtcatattcaccggattcatgggatttataatagaacaatatataaatcctattgtcaggaactcaaagcatcctttgaaaggcgatcttctatatgctattgaaagagtgttgaagctttcagttccaaatttatatgtgtggctctgcatgttctactgcttcttccacctttggttaaacatattggcagagcttctctgcttcggggatcgtgaattctacaaagattggtggaatgcaaaaagtgtgggagattactggagaatgtggaatatgcctgttcataaatggatggttcgacatatatacttcccgtgcttgcgcagcaagataccaaagacactcgccattatcattgctttcctagtctctgcagtctttcatgagctatgcatcgcagttccttgtcgtctcttcaagctatgggcttttcttgggattatgtttcaggtgcctttggtcttcatcacaaactatctacaggaaaggtttggctcaacggtggggaacatgatcttctggttcatcttctgcattttcggacaaccgatgtgtgtgcttctttattaccacgacctgatgaaccgaaaaggatcgatgtcatga

SEQ ID NO: 75 - protein, 520 aa, Arabidopsis thaliana
MAILDSAGVTTVTENGGGEFVDLDRLRRRKSRSDSSNGLLLSGSDNNSPSDDVGAPADVRDRIDSVVNDDAQGTANLAGDNNGGGDNNGGGRGGGEGRGNADATFTYRPSVPAHRRARESPLSSDAIFKQSHAGLFNLCVVVLIAVNSRLIIENLMKYGWLIRTDFWFSSRSLRDWPLFMCCISLSIFPLAAFTVEKLVLQKYISEPVVIFLHIIITMTEVLYPVYVTLRCDSAFLSGVTLMLLTCIVWLKLVSYAHTSYDIRSLANAADKANPEVSYYVSLKSLAYFMVAPTLCYQPSYPRSACIRKGWVARQFAKLVIFTGFMGFIIEQYINPIVRNSKHPLKGDLLYAIERVLKLSVPNLYVWLCMFYCFFHLWLNILAELLCFGDREFYKDWWNAKSVGDYWRMWNMPVHKWMVRHIYFPCLRSKIPKTLAIIIAFLVSAVFHELCIAVPCRLFKLWAFLGIMFQVPLVFITNYLQERFGSTVGNMIFWFIFCIFGQPMCVLLYYHDLMNRKGSMS

SEQ ID NO: 76 - protein, 9 aa, Artificial Sequence
  Elongase consenus domain 7
VDTRKGAYR

SEQ ID NO: 77 - protein, 9 aa, Artificial Sequence
  Elongase consenus domain 8
FIHTIMYTY

SEQ ID NO: 78 - DNA, 28 bp, Artificial Sequence
  Oligonucleotide primer
  misc_feature (20)..(20): n is a, c, g, or t
  misc_feature (23)..(23): n is a, c, g, or t
tggtggacacaaggaagggngcntaymg

SEQ ID NO: 79 - DNA, 27 bp, Artificial Sequence
  Oligonucleotide primer
gtaggtgtacatgatggtrtgdatraa

SEQ ID NO: 80 - DNA, 24 bp, Artificial Sequence
  Oligonucleotide primer
gtccttgctccagggcttccacca

SEQ ID NO: 81 - DNA, 36 bp, Artificial Sequence
  Oligonucleotide primer
atttaggtgacactatagtttttttttttttttttt

SEQ ID NO: 82 - DNA, 23 bp, Artificial Sequence
  Oligonucleotide primer
ttccagaacgagggcatctacgt

SEQ ID NO: 83 - DNA, 25 bp, Artificial Sequence
  Oligonucleotide primer
ttgggtgatctgcatgagcgtgatg

SEQ ID NO: 84 - DNA, 26 bp, Artificial Sequence
  Oligonucleotide primer
cgaatacttgaagagcttgttggaga

SEQ ID NO: 85 - DNA, 25 bp, Artificial Sequence
  Oligonucleotide primer
gggctacgagctggcagatgaagca

SEQ ID NO: 86 - DNA, 25 bp, Artificial Sequence
  Oligonucleotide primer
gaaaaaatggttgcgccacccatca

SEQ ID NO: 87 - DNA, 27 bp, Artificial Sequence
  Oligonucleotide primer
tcactacttcttcttcttgcccgcggc

SEQ ID NO: 88 - DNA, 21 bp, Artificial Sequence
  Oligonucleotide primer
ttccggtactcagcggtggcg

SEQ ID NO: 89 - DNA, 17 bp, Artificial Sequence
  Oligonucleotide primer
caggaaacagctatgac

SEQ ID NO: 90 - DNA, 20 bp, Artificial Sequence
  Oligonucleotide primer
acgtagatgccctcgttctg

SEQ ID NO: 91 - DNA, 26 bp, Artificial Sequence
  Oligonucleotide primer
caccgaatggcgactgaagggatgcc

SEQ ID NO: 92 - DNA, 27 bp, Artificial Sequence
  Oligonucleotide primer
ctactcggttttcatgcggttgctgga

SEQ ID NO: 93 - DNA, 819 bp, Pavlova pinguis
atggttgcgccacccatcacgctcgagtggctgctttcgccgaagctcaaggatgcagtgttcggtggggaggtgctctacttctccattgcctacctgtttcttgcgcccattttgaagcgcaccccgttggtggacacgcggaagggcgcgtataagagtggtatgatcgcgtacaacgtgatcatgtgcgtgttctcgctggtgtgcttcatctgccagctcgcagccctgggctatgacatgggctacttgcagtgggtgcgtgacctcacaggggacgagattgtccccctctaccaggacgtgtccccgtcccccgccttctccaacaagctcttcaagtattcgtctattgccttccactactccaagtatgttgagtacatggacaccgcatggctggtgatgaagggcaagcccgtgtccttgctccagggcttccaccactttggcgccgcctgggacacctactttggcatcaccttccagaacgagggcatctacgtgttcgtggtgctcaacgccttcatccacacgatcatgtacgcatactacgcggccactgcggcgggtctcaagttctcactgaagttcgtcatcacgctcatgcagatcacccaattcaacgtgggcttcgtaatggtgtatcactacatcaccctggagtacttccgcaactcaccggagctcgtcttctcctaccttttcaactatgcgtacgtctgcacggttctcctcctcttcatgcagttcttctacatggacaactttggcaagaagaaggccgctgccgccgcgggcaagaagaagaagtag

SEQ ID NO: 94 - protein, 272 aa, Pavlova pinguis
MVAPPITLEWLLSPKLKDAVFGGEVLYFSIAYLFLAPILKRTPLVDTRKGAYKSGMIAYNVIMCVFSLVCFICQLAALGYDMGYLQWVRDLTGDEIVPLYQDVSPSPAFSNKLFKYSSIAFHYSKYVEYMDTAWLVMKGKPVSLLQGFHHFGAAWDTYFGITFQNEGIYVFVVLNAFIHTIMYAYYAATAAGLKFSLKFVITLMQITQFNVGFVMVYHYITLEYFRNSPELVFSYLFNYAYVCTVLLLFMQFFYMDNFGKKKAAAAAGKKKK

SEQ ID NO: 95 - DNA, 840 bp, Pavlova salina
atggcgactgaagggatgccggcgataacgctggactggctgctctcgcccgggctgaaggatgccgtaattggcggggaggtgctctacttttcgcttgggtatctgctgctcgagcccatcctcaagcgctcaccgtttgtggacaagcgcaagggcgcataccgcaacggcatgatcgcgtacaacatcctcatgtgcggtttctcgctggtatgcttcgtgtgccagatggcggcgctcggccttgatcgcggccacctgcagtttgtccgcgacctcacgggcgacagcgtggtgcagctctaccaggacgtgagcccatcccctgcattcgcgaacaagctcttccggtactcagcggtggcgttccactactcaaagtacgtggagtacatggacacagcgtggcttgtgctgaagggcaagcccgtctcgttcctgcagggcttccaccacttcggcgccgcgtgggacacctactttggcatcacgtttcagaacgagggcacctacgtctttgtgctgctcaacgcattcatccacacaatcatgtacacctactacggcgcgacggcagcgggcatcaaaatctcgatgaagccgctgatcaccctcatgcagatcacgcagttcctgctgggcttcgcgctcgtctacccgtacattgacctcggctacttccgtgcgtcgcccgagctcgtgtggagctacctgttcaactatgcgtacgtactcatggtgctcttcctcttcatgcgcttcttctaccacgacaactttagcaagcacaagccaatctcgcgcatcgactccagcaaccgcatgaaaaccgagtag

SEQ ID NO: 96 - protein, 279 aa, Pavlova salina
MATEGMPAITLDWLLSPGLKDAVIGGEVLYFSLGYLLLEPILKRSPFVDKRKGAYRNGMIAYNILMCGFSLVCFVCQMAALGLDRGHLQFVRDLTGDSVVQLYQDVSPSPAFANKLFRYSAVAFHYSKYVEYMDTAWLVLKGKPVSFLQGFHHFGAAWDTYFGITFQNEGTYVFVLLNAFIHTIMYTYYGATAAGIKISMKPLITLMQITQFLLGFALVYPYIDLGYFRASPELVWSYLFNYAYVLMVLFLFMRFFYHDNFSKHKPISRIDSSNRMKTE

SEQ ID NO: 97 - protein, 172 aa, Tomato bushy stunt virus
MERAIQGNDAREQANSERWDGGSGGTTSPFKLPDESPSWTEWRLHNDETNSNQDNPLGFKESWGFGKVVFKRYLRYDRTEASLHRVLGSWTGDSVNYAASRFFGFDQIGCTYSIRFRGVSITVSGGSRTLQHLCEMAIRSKQELLQLAPIEVESNVSRGCPEGTETFEKESE

SEQ ID NO: 98 - protein, 116 aa, Tomato yellow leaf curl virus
MWDPLLNEFPESVHGFRCMLAIKYLQSVEETYEPNTLGHDLIRDLISVVRARDYVEATRRYNHFHARLEGSPKAELRQPIQQPCCCPHCPRHKQATIMDVQAHVPEAQNIQNVSKP

SEQ ID NO: 99 - protein, 351 aa, Turnip crinkle virus
MENDPRVRKFASEGAQWAIKWQKKGWSSLTSRQKQTARAAMGIKLSPVAQPVQKVTRLSAPVALAYREVSTQPRVSTARDGITRSGSELITTLKKNTDTEPKYTTAVLNPSEPGTFNQLIKEAAQYEKYRFTSLRFRYSPMSPSTTGGKVALAFDRDAAKPPPNDLASLYNIEGCVSSVPWTGFILTVPTDSTDRFVADGISDPKLVNFGKLIMATYGQGANDAAQLGEVRVEYTVQLKNRTGSTSDAQIGDFAGVKDGPRLVSWSKTKGTAGWEHDCHFLGTGNFSLTLFYEKAPVSGLENADASDFSVLGEAAAGSVQWAGVKVAERGQSVKMVTTEEQPRGKWQALRI

SEQ ID NO: 100 - protein, 303 aa, Pea mosaic virus
MHGIEQPQLPLDYVHRCASTSFLLASLDGLLSEARELSGPLALITSSYYLLVSIALCWAIPGSFWYRPGCWLQPVSGRNLIFCGPTEALQRFRLYAARLGLVLSENCPRHGQSAAITLQSYWALPNNIWMDMAQLDLLTFSMPIANTFAYLADCEARFPPIVEGVGSAYYVPTLLGLTHQDPRLYLALRRRNLDLSGEPHRVRPGVLESMALLCSSVRSTSRSRQIPPLYGSVLHHVLGLAERDCILFDTDSNYSSYTHRVLEQDRNRADQSLFSIDLEYVHDLELIALGYSDEDDEDLDNFF

SEQ ID NO: 101 - protein, 256 aa, Cereal yellow dwarf virus
MFIAQPCGRVLVFDVASRTPSFFTRYSVELSLRVLDPFFTRAVTDFRYTQNEIDLFCVSLGFLLPILLTGESYSWRGHLNLPLSYTELLVRWGLAVGYFPTFSTDGDIRQNPELRIDLSTMSTRSFYEQFLLRYNTSGLAKAIVGQQECFQSGMESFKRFLHYRLTCFESCLPRPRWESPLAPGPYLDRAFEATLLGRMVGHNQLLFTGLSSDITRYYNELVVEGVPVAFWDAAGITLHHAGEEYFSNSYIQKILQ

SEQ ID NO: 102 - DNA, 519 bp, Tomato bushy stunt virus
atggaacgagctatacaaggaaacgacgctagggaacaagctaacagtgaacgttgggatggaggatcaggaggtaccacttctcccttcaaacttcctgacgaaagtccgagttggactgagtggcggctacataacgatgagacgaattcgaatcaagataatccccttggtttcaaggaaagctggggtttcgggaaagttgtatttaagagatatctcagatacgacaggacggaagcttcactgcacagagtccttggatcttggacgggagattcggttaactatgcagcatctcgatttttcggtttcgaccagatcggatgtacctatagtattcggtttcgaggagttagtatcaccgtttctggagggtcgcgaactcttcagcatctctgtgagatggcaattcggtctaagcaagaactgctacagcttgccccaatcgaagtggaaagtaatgtatcaagaggatgccctgaaggtactgagaccttcgaaaaagaaagcgagtaa

SEQ ID NO: 103 - DNA, 351 bp, Tomato yellow leaf curl virus
atgtgggatccacttctaaatgaatttcctgaatctgttcacggatttcgttgtatgttagctattaaatatttgcagtccgttgaggaaacttacgagcccaatacattgggccacgatttaattagggatcttatatctgttgtaagggcccgtgactatgtcgaagcgaccaggcgatataatcatttccacgcccgcctcgaaggttcgccgaaggctgaacttcgacagcccatacagcagccgtgctgctgtccccattgtccaaggcacaaacaagcgacgatcatggacgtacaggcccatgtaccggaagcccagaatatacagaatgtatcgaagccctga

SEQ ID NO: 104 - DNA, 1056 bp, Turnip crinkle virus
atggaaaatgatcctagagtccgaaagttcgcatccgagggcgcccaatgggcgataaagtggcagaagaagggctggtcatccctaaccagcagacagaaacagaccgcccgcgcagcgatggggatcaagctctcccctgtggcgcaacctgtgcagaaagtgactcgactgagtgctccggtggctctcgcctaccgcgaggtttccacccagcctcgggtttctactgccagggacggcataaccagaagcggttctgaactgatcacaaccctgaagaagaacactgacactgaacctaagtacaccacagctgtgcttaacccaagcgaacccggaacattcaaccaactcatcaaggaggcggcccagtatgaaaaataccgattcacgtcactcagatttaggtactctcccatgagcccttcaaccaccgggggcaaggtggctctggcattcgaccgagacgctgccaaacctccgcccaacgacctcgcttccctctacaacatagagggttgtgtatctagcgtgccctggacagggtttattttgaccgtcccaacagattctactgaccgctttgtggcggatggtatcagcgatccaaagcttgtcaatttcggcaagctcatcatggccacctatggccaaggagccaatgatgccgcccaactcggtgaagtgcgagtcgagtacaccgtgcagctcaagaacagaactggctcaaccagcgacgcccagattggggacttcgcgggtgttaaggacggacccaggttggtctcgtggtccaagaccaagggaacagctgggtgggagcacgattgtcattttctcggaaccggaaacttctcgttgacactgttctacgagaaggcgcccgtttcggggctagaaaacgcagacgcctctgacttctcggtcctgggagaagccgcagcaggtagtgtccaatgggctggagtgaaggtagcagaaaggggacaaagcgtgaaaatggtcacaactgaggagcagccaaggggaaaatggcaagcactcaggatttag

SEQ ID NO: 105 - DNA, 912 bp, Pea mosaic virus
atgcacggaattgagcagcctcaactaccgctagattacgttcaccgttgcgcatcaacctccttcttgctcgcatcactagatggcctcctttctgaagcccgtgaactctcagggcctctggctctcattacttctagctattacttacttgtttctattgccctctgctgggcaatccctggatccttctggtataggcctggctgctggttgcagccagtctcagggcggaatctcatcttttgcggccctaccgaggccttgcaacgattccgtctgtacgctgccagacttgggttggtcctgtcagagaactgcccaagacacggccaatcagcagcaatcacccttcaatcatactgggcacttcctaacaacatctggatggacatggcccaattggacttgctcaccttctcaatgccaattgctaatacatttgcctacttggcagattgtgaagcaagatttcctcctattgttgaaggagtgggatctgcttactatgtgccaacgctgctcggacttactcaccaagaccccaggctttatcttgcgcttcgcaggagaaaccttgatcttagtggcgaacctcatagagttcgtcctggtgtcctggagtctatggctttgctctgttctagtgtacgtagcacaagccgttccaggcaaattcctcctttatatggcagcgttttgcaccacgttttgggcctggccgagagagactgcatcctctttgatacggatagtaactactcctcttacactcatcgggttcttgaacaagaccggaatcgggctgatcagtcattgtttagcattgacttggaatatgttcatgacctggagcttattgccctgggttactctgatgaagatgatgaagatcttgataacttcttctag

SEQ ID NO: 106 - DNA, 771 bp, Cereal yellow dwarf virus
atgttcatcgcccaaccttgcgggcgagttcttgtgttcgacgtcgcctcccgcacgccatcgttcttcactcgttatagtgttgaactctcgctccgtgttctagacccattcttcacgcgagcagtaacagatttccgatacacccaaaatgaaatcgatttattttgtgtgtctcttggctttctgttgccaattctcctcacaggagaatcttactcttggcgcggtcacctcaacctccccctttcttacaccgaattacttgttcgatgggggctcgcagtggggtacttccctaccttctccactgatggtgacattcgacagaacccagaactccgcatcgacctgtccaccatgtcaacccgctctttctacgagcagttcctactcagatataacacgagtgggttggcaaaagctatcgtcggacagcaagagtgctttcaaagcggcatggagtcttttaaaagattcctacactaccgcctcacgtgctttgaaagctgccttccacgacctcgttgggaaagtcctttggctcctggtccttatctggacagggcttttgaggcaactcttctcggccgtatggtcggtcataaccaactactctttaccggtttgtcttctgatatcactaggtattataacgagttggttgtggaaggcgtgccggtggctttttgggacgctgccggcattactttgcatcacgctggtgaagaatatttttcgaattcttacattcaaaagattcttcaatga

SEQ ID NO: 107 - DNA, 1005 bp, Micromonas CCMP1545
atgaccgctgctccagcttctgctagagatcctgctcttgctactggatctggatctctttacaaccacctcatgatgttcgcttggcttggagttgttcatgctgttgttgctcttgttgctgttgcttgctacttccttcctcatcctgttgctacttgtgctatcgctctcgttgctcttgctgctcttactcctgttactactcctcatcctgcttggggacttgctatcgctagagctatcactaaggctgctgtgagatacttccctcttactatggaatgggaggatgagagagcttaccttgacgctgctgctaagggtgttcctgctgttatcggacttgagcctcattctgttctccctttgtctatcgttgctttcggaaactacttcttcttcaccgaatctacacctgagtgcgtgagaaactctagagctttggctactggaaccatcttcgttatccctgttcttaagcacctttggtcttggcttggaatggatgctatctctaggcgtgctatgaagactcttctcgatgatggaagatctgttctcatcatccctggtggagttgctgagtgccttcaaatgaggcctggtgttgagactatctacctcaagaagaggttcggattcgttaagcttgctatccaaaccggtgcttctcttgttcctgctttcactttcggacagaccagatcttactcttactggcgtcttggacctcctcttgttcctcatgttgttgctgaggttttcgctagagcttgtagagttgctcctatggttttctggggaaagtggggatctcctatccctaacatggttcctatgcacactgttgttggaaagcctatccctgttaagaagcagtctgagccttctaacgagtacgttcaagagaagctcaacgagttcgttgctgctatggaatctctttacgctagacacaagggaaagcacggatacgctgagtctactctcgttgttctttga

SEQ ID NO: 108 - protein, 334 aa, Micromonas CCMP1545
MTAAPASARDPALATGSGSLYNHLMMFAWLGVVHAVVALVAVACYFLPHPVATCAIALVALAALTPVTTPHPAWGLAIARAITKAAVRYFPLTMEWEDERAYLDAAAKGVPAVIGLEPHSVLPLSIVAFGNYFFFTESTPECVRNSRALATGTIFVIPVLKHLWSWLGMDAISRRAMKTLLDDGRSVLIIPGGVAECLQMRPGVETIYLKKRFGFVKLAIQTGASLVPAFTFGQTRSYSYWRLGPPLVPHVVAEVFARACRVAPMVFWGKWGSPIPNMVPMHTVVGKPIPVKKQSEPSNEYVQEKLNEFVAAMESLYARHKGKHGYAESTLVVL

SEQ ID NO: 109 - DNA, 17 bp, Artificial Sequence
  Transfer nucleic acid border sequence
  misc_feature (2)..(2): n is a, c, g, or t
  misc_feature (6)..(6): n is a, c, g, or t
  misc_feature (10)..(15): n is a, c, g, or t
angatntatnnnnnngt

SEQ ID NO: 110 - DNA, 25 bp, Artificial Sequence
  Transfer nucleic acid border sequence
tgacaggatatattggcgggtaaac

SEQ ID NO: 111 - DNA, 25 bp, Artificial Sequence
  Transfer nucleic acid border sequence
tggcaggatatattgtggtgtaaac

SEQ ID NO: 112 - DNA, 25 bp, Artificial Sequence
  Transfer nucleic acid border sequence
tggcaggatatataccgttgtaatt

SEQ ID NO: 113 - DNA, 25 bp, Artificial Sequence
  Transfer nucleic acid border sequence
cggcaggatatattcaattgtaatt

SEQ ID NO: 114 - DNA, 25 bp, Artificial Sequence
  Transfer nucleic acid border sequence
tggtaggatatataccgttgtaatt

SEQ ID NO: 115 - DNA, 25 bp, Artificial Sequence
  Transfer nucleic acid border sequence
tggcaggatatatggtactgtaatt

SEQ ID NO: 116 - DNA, 25 bp, Artificial Sequence
  Transfer nucleic acid border sequence
  misc_feature (1)..(1): y = c or t
  misc_feature (3)..(3): r = a or g
  misc_feature (4)..(4): y = c or t
  misc_feature (14)..(14): w = a or t
  misc_feature (15)..(15): s = c or g
  misc_feature (16)..(16): n is a, c, g, or t
  misc_feature (17)..(17): v = a, c or g
  misc_feature (18)..(18): b = c, g or t
  misc_feature (19)..(19): k = g or t
  misc_feature (24)..(24): w = a or t
  misc_feature (25)..(25): y = c or t
ygryaggatatatwsnvbkgtaawy

SEQ ID NO: 117 - DNA, 25 bp, Artificial Sequence
  Transfer nucleic acid border sequence
cggcaggatatatcctgatgtaaat

SEQ ID NO: 118 - DNA, 25 bp, Artificial Sequence
  Transfer nucleic acid border sequence
tggcaggagttattcgagggtaaac

SEQ ID NO: 119 - DNA, 25 bp, Artificial Sequence
  Transfer nucleic acid border sequence
tgacaggatatatcgtgatgtcaac

SEQ ID NO: 120 - DNA, 25 bp, Artificial Sequence
  Transfer nucleic acid border sequence
gggaagtacatattggcgggtaaac

SEQ ID NO: 121 - DNA, 25 bp, Artificial Sequence
  Transfer nucleic acid border sequence
ttacaggatatattaatatgtatga

SEQ ID NO: 122 - DNA, 25 bp, Artificial Sequence
  Transfer nucleic acid border sequence
taacatgatatattcccttgtaaat

SEQ ID NO: 123 - DNA, 25 bp, Artificial Sequence
  Transfer nucleic acid border sequence
tgacaggatatatggtaatgtaaac

SEQ ID NO: 124 - DNA, 25 bp, Artificial Sequence
  Transfer nucleic acid border sequence
tggcaggatatataccgatgtaaac

SEQ ID NO: 125 - DNA, 1395 bp, Artificial Sequence
  Codon-optimized nucleotide sequence for production in plants of SEQ ID NO:7
atgtgtcctcctaagaccgatggaagatcttctcctagatctcctctcaccaggtctaagtcatctgctgaggctcttgatgctaaggatgcttctaccgctcctgttgatcttaagacccttgagcctcatgaacttgctgctaccttcgagactagatgggttagggttgaggatgttgagtacgacgtgaccaacttcaaacatcctggtggaagcgtgatcttctacatgcttgctaacactggtgctgatgctactgaggctttcaaagaatttcacatgcgtagcctcaaggcttggaagatgcttagagctttgccttctagacctgctgagatcaagagatctgagtctgaggatgctcctatgcttgaggatttcgctaggtggagagctgaacttgagagggacggattcttcaagccttctatcacccatgttgcttaccgtcttttggagcttcttgctactttcgctcttggaaccgctcttatgtacgctggataccctatcattgctagcgttgtgtacggtgctttcttcggagctagatgtggatgggttcaacatgagggtggacacaactctcttaccggatctgtgtacgtggataagagacttcaggctatgacttgcggattcggactttctaccagcggagagatgtggaaccagatgcataacaagcaccatgctacccctcagaaagttagacacgacatggatcttgataccactcctgctgtggctttcttcaacaccgctgtggaggataatagacctaggggattctctagagcttgggctagacttcaagcttggaccttcgttcctgttacttctggacttctcgttcaggctttctggatctacgttctccatcctagacaggtgctcaggaagaagaactacgaggaagcttcttggatgctcgtttctcacgttgttagaaccgctgttatcaagcttgctaccggatactcttggcctgttgcttactggtggttcactttcggaaactggatcgcttacatgtacctcttcgctcacttctctacttctcacactcacctccctgttgttccatctgacaagcaccttagctgggttaactacgctgttgatcacaccgttgacatcgatccttctcgtggatacgttaactggcttatgggataccttaactgccaggttatccaccatctcttccctgatatgcctcaattcagacagcctgaggtgtcaagaagattcgtccctttcgctaagaagtggggactcaactacaaggtgctctcttactacggtgcttggaaggctactttcagcaacctcgacaaagttggacagcactactacgttaacggaaaggctgagaaggctcactgatga

SEQ ID NO: 126 - DNA, 870 bp, Artificial Sequence
  Codon-optimized nucleotide sequence for production in plants of SEQ ID NO:3
atggaatttgctcaacctctcgttgctatggctcaagagcagtacgctgctatcgatgctgttgttgctcctgctatcttctctgctaccgactctattggatggggactcaagcctatctcttctgctactaaggatctccctctcgttgaatctcctacccctcttatcctttctctcctcgcttacttcgctatcgttggttctggactcgtttaccgtaaagtgttccctagaaccgttaagggacaggatcctttccttctcaaggctcttatgctcgctcacaacgttttccttatcggactcagcctttacatgtgcctcaagctcgtttacgaggcttacgtgaacaagtactccttctggggaaacgcttacaaccctgctcaaaccgagatggctaaggtgatctggatcttctacgtgtccaagatctacgagttcatggacaccttcatcatgcttctcaagggaaacgttaaccaggtttccttcctccatgtttaccaccacggatctatctctggaatctggtggatgatcacttatgctgctccaggtggagatgcttacttctctgctgctctcaactcttgggttcatgtgtgcatgtacacctactacttcatggctgctgttcttcctaaggacgaaaagaccaagagaaagtacctttggtggggaagataccttacccagatgcaaatgttccagttcttcatgaaccttctccaggctgtttacctcctctactcttcttctccttaccctaagttcattgctcaactcctcgttgtttacatggttaccctcctcatgcttttcggaaacttctactacatgaagcaccacgcttctaagtgataa

SEQ ID NO: 127 - DNA, 1281 bp, Artificial Sequence
  Codon-optimized nucleotide sequence for production in plants of SEQ ID NO:25
atgcctcctagggactcttactcttacgctgctcctccttctgctcaacttcacgaggttgacactcctcaagagcacgacaagaaagagcttgttatcggagatagggcttacgatgtgaccaacttcgttaagagacaccctggtggaaagatcattgcttaccaagtgggaactgatgctaccgatgcttacaagcagttccatgtgagatctgctaaggctgacaagatgctcaagtctctcccttctagacctgttcacaagggatactctcctagaagagctgatcttatcgctgacttccaagagttcactaagcaacttgaggctgagggaatgttcgaaccttctctccctcatgttgcttaccgtcttgctgaggttatcgctatgcatgttgctggtgctgctcttatctggcacggatacactttcgctggaatcgctatgcttggagttgttcagggaagatgcggatggcttatgcatgagggtggacactactctcttaccggaaacattgctttcgatagggctatccaagttgcttgttacggacttggatgcggaatgtctggtgcttggtggagaaaccagcataacaagcaccatgctactcctcaaaagctccagcacgatgttgatcttgataccctccctctcgttgctttccatgagagaatcgctgctaaggttaagtctcctgctatgaaggcttggctctccatgcaagctaaactcttcgctcctgttaccactcttcttgttgctcttggatggcagctttaccttcaccctagacacatgctcagaactaagcactacgacgagcttgctatgcttggtatcagatacggacttgtgggataccttgctgctaactacggtgctggatacgttcttgcttgctaccttctctacgttcagcttggagctatgtacatcttctgcaacttcgctgtttctcacactcatctccctgttgttgagcctaacgagcatgctacttgggttgagtacgctgctaaccacactactaactgctctccatcttggtggtgtgattggtggatgagctacctcaactaccagatcgagcatcacctttacccttctatgcctcagttcaggcatcctaagatcgctcctagagtgaagcaactcttcgagaagcacggacttcactacgatgtgcgtggatacttcgaggctatggctgatactttcgctaacctcgataacgttgctcatgctcctgagaagaaaatgcaatgatga

SEQ ID NO: 128 - DNA, 807 bp, Artificial Sequence
  Codon-optimized nucleotide sequence for production in plants of SEQ ID NO:5
atggcttctatcgctatccctgctgctcttgctggaactcttggatacgtgacctacaacgtggctaaccctgatattcctgcttctgagaaggttccagcttacttcatgcaagtggagtactggggacctactatcggaactatcggttacctcctcttcatctacttcggaaagcgtatcatgcaaaacagaagccagcctttcggacttaagaacgctatgctcgtgtacaacttctaccagaccttcttcaacagctactgcatctacctcttcgttacctctcatagggctcagggacttaaagtttggggaaacatccctgatatgaccgctaactcttggggaatctctcaggttatctggctccactacaacaacaagtacgtggagcttctcgataccttcttcatggtgatgaggaagaagttcgaccagctttctttccttcacatctaccaccacactcttctcatctggtcatggttcgtggttatgaagctcgagcctgttggagattgctacttcggatctagcgttaacaccttcgtgcacgtgatcatgtactcttactacggacttgctgctcttggagttaactgcttctggaagaagtacatcacccagatccagatgcttcagttctgtatctgcgcttctcactctatctacaccgcttacgttcagaacactgctttctggcttccttaccttcagctctgggtgatggttaacatgttcgtgctcttcgctaacttctaccgtaaaaggtacaagagcaagggtgctaagaagcagtgataa

SEQ ID NO: 129 - DNA, 1347 bp, Artificial Sequence
  Codon-optimized nucleotide sequence for production in plants of SEQ ID NO:72
atgcctccatctgctgctaaacagatgggagcttctactggtgttcacgctggtgttaccgattcttctgctttcaccagaaaggatgtggctgatagacctgatcttaccatcgttggtgactctgtgtacgatgctaaggctttcagatctgagcatcctggtggtgctcatttcgtttcactcttcggaggaagagatgctactgaggctttcatggaataccacagaagagcttggcctaagtctaggatgtctaggttccatgttggatctcttgcttctaccgaggaacctgttgctgctgatgagggataccttcagctttgtgctaggatcgctaagatggtgccttctgtgtcatctggattcgctccagcttcttactgggttaaggctggacttatcctcggatctgctatcgctcttgaggcttacatgctctacgctggaaagagacttctcccttctatcgttcttggatggctcttcgctcttatcggacttaacatccagcatgacgctaaccatggtgctttgtctaagtctgctagcgttaaccttgctcttggactttgtcaggattggatcggaggatctatgatcctttggctccaagagcatgttgttatgcaccacctccacaccaacgatgttgataaggaccctgatcaaaaggctcatggtgctcttagactcaagcctaccgatgcttggtcacctatgcattggcttcagcacctttaccttctccctggtgaaactatgtacgctttcaagctcctcttcctcgatatctctgagcttgtgatgtggagatgggagggtgaacctatctctaagctcgctggatacctcttcatgccttctcttctcctcaagcttaccttctgggctagattcgttgctcttcctctttacctcgctccttctgttcatactgctgtgtgtatcgctgctactgttatgaccggaagcttctaccttgctttcttcttcttcatcagccacaacttcgagggtgttgcttctgttggacctgatggatctatcacctctatgaccaggggagcttctttccttaagaggcaggctgagacttcttctaatgtgggaggacctcttcttgctactcttaacggtggactcaactaccaaatcgagcaccaccttttccctagagttcaccacggattctaccctagacttgctcctcttgtgaaggctgaacttgaggctagaggaatcgagtacaagcactaccctaccatctggtctaacctcgcttctaccctcagacatatgtacgctcttggaagaaggcctagatctaaggctgagtgatga